European Patent Specification EP 3 341 016 B9, published September 27, 2023. Title: METHODS AND COMPOSITIONS FOR IMMUNE PROTECTION AGAINST EXTRA-INTESTINAL PATHOGENIC E. COLI. Applicant: GlycoVaxyn AG Janssen Pharmaceuticals, Inc. The sequence listing filed with the application follows.

SEQUENCE LISTING (3 sequences)

SEQ ID NO: 1 - protein, 652 aa, Artificial Sequence
  Detoxified EPA protein comprising 4 optimized N-glycosylation sequences
GSGGGDQNATGSGGGKLAEEAFDLWNECAKACVLDLKDGVRSSRMSVDPAIADTNGQGVLHYSMVLEGGNDALKLAIDNALSITSDGLTIRLEGGVEPNKPVRYSYTRQARGSWSLNWLVPIGHEKPSNIKVFIHELNAGNQLSHMSPIYTIEMGDELLAKLARDATFFVRAHESNEMQPTLAISHAGVSVVMAQAQPRREKRWSEWASGKVLCLLDPLDGVYNYLAQQRCNLDDTWEGKIYRVLAGNPAKHDLDIKDNNNSTPTVISHRLHFPEGGSLAALTAHQACHLPLEAFTRHRQPRGWEQLEQCGYPVQRLVALYLAARLSWNQVDQVIRNALASPGSGGDLGEAIREQPEQARLALTLAAAESERFVRQGTGNDEAGAASADVVSLTCPVAKDQNRTKGECAGPADSGDALLERNYPTGAEFLGDGGDVSFSTRGTQNWTVERLLQAHRQLEERGYVFVGYHGTFLEAAQSIVFGGVRARSQDLDAIWRGFYIAGDPALAYGYAQDQEPDARGRIRNGALLRVYVPRWSLPGFYRTGLTLAAPEAAGEVERLIGHPLPLRLDAITGPEEEGGRVTILGWPLAERTVVIPSAIPTDPRNVGGDLDPSSIPDKEQAISALPDYASQPGKPPREDLKLGSGGGDQNAT

SEQ ID NO: 2 - protein, 3 aa, Artificial Sequence
  N-glycosylation consensus sequence
  any amino acid (except Pro) (2)..(2)
  Ser or Thr (3)..(3)
NXX

SEQ ID NO: 3 - protein, 5 aa, Artificial Sequence
  N-glycosylation consensus sequence
  Asp or Glu (1)..(1)
  any natural amino acid except Pro (2)..(2)
  any natural amino acid except Pro (4)..(4)
  Ser or Thr (5)..(5)
XXNXX